European Patent Application EP 4 628 507 A1, published October 8, 2025. Title: CLDN18.2/4-1BB结合蛋白及其医药用途. Applicant: 江苏恒瑞医药股份有限公司. Application WO. The sequence listing filed with the application follows.

SEQUENCE LISTING (107 sequences)

SEQ ID NO: 1 - protein, 448 aa, synthetic construct
  source 1..448: note = Urelumab
QVQLQQWGAGLLKPSETLSLTCAVYGGSFSGYYWSWIRQSPEKGLEWIGEINHGGYVTYNPSLESRVTISVDTSKNQFSLKLSSVTAADTAVYYCARDYGPGNYDWYFDLWGRGTLVTVSSASTKGPSVFPLAPCSRSTSESTAALGCLVKDYFPEPVTVSWNSGALTSGVHTFPAVLQSSGLYSLSSVVTVPSSSLGTKTYTCNVDHKPSNTKVDKRVESKYGPPCPPCPAPEFLGGPSVFLFPPKPKDTLMISRTPEVTCVVVDVSQEDPEVQFNWYVDGVEVHNAKTKPREEQFNSTYRVVSVLTVLHQDWLNGKEYKCKVSNKGLPSSIEKTISKAKGQPREPQVYTLPPSQEEMTKNQVSLTCLVKGFYPSDIAVEWESNGQPENNYKTTPPVLDSDGSFFLYSRLTVDKSRWQEGNVFSCSVMHEALHNHYTQKSLSLSLGK

SEQ ID NO: 2 - protein, 216 aa, synthetic construct
  source 1..216: note = Urelumab
EIVLTQSPATLSLSPGERATLSCRASQSVSSYLAWYQQKPGQAPRLLIYDASNRATGIPARFSGSGSGTDFTLTISSLEPEDFAVYYCQQRSNWPPALTFCGGTKVEIKRTVAAPSVFIFPPSDEQLKSGTASVVCLLNNFYPREAKVQWKVDNALQSGNSQESVTEQDSKDSTYSLSSTLTLSKADYEKHKVYACEVTHQGLSSPVTKSFNRGEC

SEQ ID NO: 3 - protein, 448 aa, synthetic construct
  source 1..448: note = IMAB362
QVQLQQPGAELVRPGASVKLSCKASGYTFTSYWINWVKQRPGQGLEWIGNIYPSDSYTNYNQKFKDKATLTVDKSSSTAYMQLSSPTSEDSAVYYCTRSWRGNSFDYWGQGTTLTVSSASTKGPSVFPLAPSSKSTSGGTAALGCLVKDYFPEPVTVSWNSGALTSGVHTFPAVLQSSGLYSLSSVVTVPSSSLGTQTYICNVNHKPSNTKVDKRVEPKSCDKTHTCPPCPAPELLGGPSVFLFPPKPKDTLMISRTPEVTCVVVDVSHEDPEVKFNWYVDGVEVHNAKTKPREEQYNSTYRVVSVLTVLHQDWLNGKEYKCKVSNKALPAPIEKTISKAKGQPREPQVYTLPPSREEMTKNQVSLTCLVKGFYPSDIAVEWESNGQPENNYKTTPPVLDSDGSFFLYSKLTVDKSRWQQGNVFSCSVMHEALHNHYTQKSLSLSPGK

SEQ ID NO: 4 - protein, 220 aa, synthetic construct
  source 1..220: note = IMAB362
DIVMTQSPSSLTVTAGEKVTMSCKSSQSLLNSGNQKNYLTWYQQKPGQPPKLLIYWASTRESGVPDRFTGSGSGTDFTLTISSVQAEDLAVYYCQNDYSYPFTFGSGTKLEIKRTVAAPSVFIFPPSDEQLKSGTASVVCLLNNFYPREAKVQWKVDNALQSGNSQESVTEQDSKDSTYSLSSTLTLSKADYEKHKVYACEVTHQGLSSPVTKSFNRGEC

SEQ ID NO: 5 - protein, 716 aa, synthetic construct
  source 1..716: note = TJ-CD4B
QVQLVQSGAEVKKPGASVKVSCKASGYTFTTYPIEWVRQAPGQRLEWMGNFHPYNDDTKYNEKFKGRVTITRDTSASTAYMELSSLRSEDTAVYYCARRAYGYPYAMDYWGQGTLVTVSSASTKGPSVFPLAPSSKSTSGGTAALGCLVKDYFPEPVTVSWNSGALTSGVHTFPAVLQSSGLYSLSSVVTVPSSSLGTQTYICNVNHKPSNTKVDKKVEPKSCDKTHTCPPCPAPELLGGPSVFLFPPKPKDTLMISRTPEVTCVVVDVSHEDPEVKFNWYVDGVEVHNAKTKPREEQYASTYRVVSVLTVLHQDWLNGKEYKCKVSNKALPAPIEKTISKAKGQPREPQVYTLPPSREEMTKNQVSLTCLVKGFYPSDIAVEWESNGQPENNYKTTPPVLDSDGSFFLYSKLTVDKSRWQQGNVFSCSVMHEALHNHYTQKSLSLSPGKGGGGSGGGGSGGGGSQSVLTQPPSASGTPGQRVTISCSGSSSNIGNNYVTWYQQLPGTAPKLLIYADSHRPSGVPDRFSGSKSGTSASLAISGLRSEDEADYYCATWDYSLSGYVFGCGTKLTVLGGGGSGGGGSGGGGSGGGGSEVQLLESGGGLVQPGGSLRLSCAASGFTFSSYDMSWVRQAPGKCLEWVSWISYSGGSIYYADSVKGRFTISRDNSKNTLYLQMNSLRAEDTAVYYCARDAQRNSMREFDYWGQGTLVTVSS

SEQ ID NO: 6 - protein, 220 aa, synthetic construct
  source 1..220: note = TJ-CD4B
DIVMTQSPDSLAVSLGERATINCKSSQSLLNAGNQKNYLTWYQQKPGQPPKLLIYRASSRESGVPDRFSGSGSGTDFTLTISSLQAEDVAVYYCQNDYIYPYTFGGGTKLEIKRTVAAPSVFIFPPSDEQLKSGTASVVCLLNNFYPREAKVQWKVDNALQSGNSQESVTEQDSKDSTYSLSSTLTLSKADYEKHKVYACEVTHQGLSSPVTKSFNRGEC

SEQ ID NO: 7 - protein, 450 aa, synthetic construct
  source 1..450: note = ADG106
EVQLVESGGGLVQPGGSLRLSCAASGFSLSTGGVGVGWIRQAPGKGLEWLALIDWADDKYYSPSLKSRLTISRDNSKNTLYLQLNSLRAEDTAVYYCARGGSDTVIGDWFAYWGQGTLVTVSSASTKGPSVFPLAPCSRSTSESTAALGCLVKDYFPEPVTVSWNSGALTSGVHTFPAVLQSSGLYSLSSVVTVPSSSLGTKTYTCNVDHKPSNTKVDKRVESKYGPPCPPCPAPEFLGGPSVFLFPPKPKDTLMISRTPEVTCVVVDVSQEDPEVQFNWYVDGVEVHNAKTKPREEQFNSTYRVVSVLTVLHQDWLNGKEYKCKVSNKGLPSSIEKTISKAKGQPREPQVYTLPPSQEEMTKNQVSLTCLVKGFYPSDIAVEWESNGQPENNYKTTPPVLDSDGSFFLYSRLTVDKSRWQEGNVFSCSVMHEALHNHYTQKSLSLSLGK

SEQ ID NO: 8 - protein, 213 aa, synthetic construct
  source 1..213: note = ADG106
DIQLTQSPSSLSASVGDRVTITCRASQSIGSYLAWYQQKPGKAPKLLIYDASNLETGVPSRFSGSGSGTDFTLTISSLQPEDFATYYCQQGYYLWTFGQGTKVEIKRTVAAPSVFIFPPSDEQLKSGTASVVCLLNNFYPREAKVQWKVDNALQSGNSQESVTEQDSKDSTYSLSSTLTLSKADYEKHKVYACEVTHQGLSSPVTKSFNRGEC

SEQ ID NO: 9 - protein, 163 aa, Homo sapiens
  source 1..163: note = 4-1BB
LQDPCSNCPAGTFCDNNRNQICSPCPPNSFSSAGGQRTCDICRQCKGVFRTRKECSSTSNAECDCTPGFHCLGAGCSMCEQDCKQGQELTKKGCKDCCFGTFNDQKRGICRPWTNCSLDGKSVLVNGTKERDVVCGPSPADLSPGASSVTPPAPAREPGHSPQ

SEQ ID NO: 10 - protein, 124 aa, synthetic construct
  source 1..124: note = C5
QVQLVESGGGLVQPGGSLRLSCSASGFTFSSYAMSWVRQAPGKGLEWVSDINSGGESTFYEDSVKGRFTISRDNAKNTLYLQMNSLKPEDTAVYYCAKHPLTFTIATMNDYDYWGQGTQVTVSS

SEQ ID NO: 11 - protein, 5 aa, synthetic construct
  source 1..5: note = CDR
SYAMS

SEQ ID NO: 12 - protein, 17 aa, synthetic construct
  source 1..17: note = CDR
DINSGGESTFYEDSVKG

SEQ ID NO: 13 - protein, 15 aa, synthetic construct
  source 1..15: note = CDR
HPLTFTIATMNDYDY

SEQ ID NO: 14 - protein, 232 aa, synthetic construct
  source 1..232: note = IgG1-Fc
EPKSADKTHTCPPCPAPELLGGPSVFLFPPKPKDTLMISRTPEVTCVVVDVEHEDPEVKFNWYVDGVEVHNAKTKPREEQYNSTYRVVSVLTVLHQDWLNGKEYKCKVSNKAFPAPIEKTISKAKGQPREPQVYTLPPSREEMTKNQVSLTCLVKGFYPSDIAVEWESNGQPENNYKTTPPVLDSDGSFFLYSKLTVDKSRWQQGNVFSCSVMHEALHNHYTQKSLSLSPGK

SEQ ID NO: 15 - protein, 232 aa, synthetic construct
  source 1..232: note = IgG1-Fc
EPKSADKTHTCPPCPAPEAAGGPSVFLFPPKPKDTLMISRTPEVTCVVVDVSHEDPEVKFNWYVDGVEVHNAKTKPREEQYASTYRVVSVLTVLHQDWLNGKEYKCKVSNKALPAPIEKTISKAKGQPREPQVYTLPPSREEMTKNQVSLTCLVKGFYPSDIAVEWESNGQPENNYKTTPPVLDSDGSFFLYSKLTVDKSRWQQGNVFSCSVMHEALHNHYTQKSLSLSPGK

SEQ ID NO: 16 - protein, 230 aa, synthetic construct
  source 1..230: note = IgG4-Fc
ESKYGPPCPPCPAPEFLGGPSVFLFPPKPKDTLMISRTPEVTCVVVDVSQEDPEVQFNWYVDGVEVHNAKTKPREEQFNSTYRVVSVLTVLHQDWLNGKEYKCKVSNKGLPSSIEKTISKAKGQPREPQVYTLPPSQEEMTKNQVSLTCLVKGFYPSDIAVEWESNGQPENNYKTTPPVLDSDGSFFLYSRLTVDKSRWQEGNVFSCSVMHEALHNHYTQKSLSLSLPGK

SEQ ID NO: 17 - protein, 356 aa, synthetic construct
  source 1..356: note = C5-Fc
QVQLVESGGGLVQPGGSLRLSCSASGFTFSSYAMSWVRQAPGKGLEWVSDINSGGESTFYEDSVKGRFTISRDNAKNTLYLQMNSLKPEDTAVYYCAKHPLTFTIATMNDYDYWGQGTQVTVSSEPKSADKTHTCPPCPAPELLGGPSVFLFPPKPKDTLMISRTPEVTCVVVDVEHEDPEVKFNWYVDGVEVHNAKTKPREEQYNSTYRVVSVLTVLHQDWLNGKEYKCKVSNKAFPAPIEKTISKAKGQPREPQVYTLPPSREEMTKNQVSLTCLVKGFYPSDIAVEWESNGQPENNYKTTPPVLDSDGSFFLYSKLTVDKSRWQQGNVFSCSVMHEALHNHYTQKSLSLSPGK

SEQ ID NO: 18 - protein, 124 aa, synthetic construct
  source 1..124: note = C5_V1
QVQLVESGGGLVQPGGSLRLSCSASGFTFSSYAMSWVRQAPGKGLEWVSDINSGGESTFYEDSVKGRFTISRDNAKNTLYLQMNSLRAEDTAVYYCARHPLTFTIATMNDYDYWGQGTLVTVSS

SEQ ID NO: 19 - protein, 124 aa, synthetic construct
  source 1..124: note = C5_V2
QVQLVESGGGLVQPGGSLRLSCSASGFTFSSYAMSWVRQAPGKGLEWVSDINSGGESTFYEDSVKGRFTISRDNAKNTLYLQMNSLRAEDTAVYYCAKHPLTFTIATMNDYDYWGQGTLVTVSS

SEQ ID NO: 20 - protein, 124 aa, synthetic construct
  source 1..124: note = C5_V3
QVQLVESGGGLVQPGGSLRLSCSASGFTFSSYAMSWVRQAPGKGLEWVSDINSGGESTFYEDSVKGRFTISRDNAKNTLYLQMNSLKPEDTAVYYCAKHPLTFTIATMNDYDYWGQGTLVTVSS

SEQ ID NO: 21 - protein, 124 aa, synthetic construct
  source 1..124: note = C5_V2-YTI
QVQLVESGGGLVQPGGSLRLSCSASGFTFSSYAMSWVRQAPGKGLEWVSDINSGGESTFYEDSVKGRFTISRDNAKNTLYLQMNSLRAEDTAVYYCAKHPLTYTIATMNDYDYWGQGTLVTVSS

SEQ ID NO: 22 - protein, 15 aa, synthetic construct
  source 1..15: note = CDR
HPLTYTIATMNDYDY

SEQ ID NO: 23 - protein, 124 aa, synthetic construct
  source 1..124: note = 34
HVQLVESGGGLVQPGGSLRLSCAASGFAFSTYAMYWVRQLPGKGLEWVSTINSDGSSTRYAGSVKGRFTISRDNAKNTLYLQLNSLKTEDTAMYYCAKGWISSPVWGDYVPPVRGQGTQVTVSA

SEQ ID NO: 24 - protein, 123 aa, synthetic construct
  source 1..123: note = 501
QVQLVESGGGLVQAGGSLRLSCTVSGFPVDAYPMGWFRQTPGKEREWLSCINWNGGRTQYGDSVKGRFTISRDNAKDTLYLQMNSLKAEDTAMYYCAALYACDSASSPSRRDWGQGTQVTVSS

SEQ ID NO: 25 - protein, 5 aa, synthetic construct
  source 1..5: note = CDR
TYAMY

SEQ ID NO: 26 - protein, 17 aa, synthetic construct
  source 1..17: note = CDR
TINSDGSSTRYAGSVKG

SEQ ID NO: 27 - protein, 15 aa, synthetic construct
  source 1..15: note = CDR
GWISSPVWGDYVPPV

SEQ ID NO: 28 - protein, 5 aa, synthetic construct
  source 1..5: note = CDR
AYPMG

SEQ ID NO: 29 - protein, 17 aa, synthetic construct
  source 1..17: note = CDR
CINWNGGRTQYGDSVKG

SEQ ID NO: 30 - protein, 14 aa, synthetic construct
  source 1..14: note = CDR
LYACDSASSPSRRD

SEQ ID NO: 31 - protein, 354 aa, synthetic construct
  source 1..354: note = VHH-2-LALA
EVQLLESGGGLVQPGGSLRLSCAASGLTFSSYNMGWVRQAPGKGLEWVASITWSGRDTFYADSVKGRFTISRDNSKNTLYLQMNSLRAEDTAVYYCAANPWPVAAPRSGTYWGQGTLVTVSSEPKSADKTHTCPPCPAPEAAGGPSVFLFPPKPKDTLMISRTPEVTCVVVDVSHEDPEVKFNWYVDGVEVHNAKTKPREEQYNSTYRVVSVLTVLHQDWLNGKEYKCKVSNKALPAPIEKTISKAKGQPREPQVYTLPPSREEMTKNQVSLTCLVKGFYPSDIAVEWESNGQPENNYKTTPPVLDSDGSFFLYSKLTVDKSRWQQGNVFSCSVMHEALHNHYTQKSLSLSPGK

SEQ ID NO: 32 - protein, 254 aa, Homo sapiens
  source 1..254: note = CD16A-V176
MWQLLLPTALLLLVSAGMRTEDLPKAVVFLEPQWYRVLEKDSVTLKCQGAYSPEDNSTQWFHNESLISSQASSYFIDAATVDDSGEYRCQTNLSTLSDPVQLEVHIGWLLLQAPRWVFKEEDPIHLRCHSWKNTALHKVTYLQNGKGRKYFHHNSDFYIPKATLKDSGSYFCRGLVGSKNVSSETVNITITQGLAVSTISSFFPPGYQVSFCLVMVLLFAVDTGLYFSVKTNIRSSTRDWKDHKFKWRKDPQDK

SEQ ID NO: 33 - protein, 233 aa, Homo sapiens
  source 1..233: note = CD16B
MWQLLLPTALLLLVSAGMRTEDLPKAVVFLEPQWYSVLEKDSVTLKCQGAYSPEDNSTQWFHNESLISSQASSYFIDAATVNDSGEYRCQTNLSTLSDPVQLEVHIGWLLLQAPRWVFKEEDPIHLRCHSWKNTALHKVTYLQNGKDRKYFHHNSDFHIPKATLKDSGSYFCRGLVGSKNVSSETVNITITQGLAVSTISSFSPPGYQVSFCLVMVLLFAVDTGLYFSVKTNI

SEQ ID NO: 34 - protein, 254 aa, Macaca fascicularis
  source 1..254: note = CD16
MWQLLLPTALLLLVSAGMRAEDLPRAVVFLEPQWYRVLEKDRVTLKCQGAYSPEDNSTRWFHNESLISSQTSSYFIAAARVNNSGEYRCQTSLSTLSDPVQLEVHIGWLLLQAPRWVFKEEESIHLRCHSWKNTLLHKVTYLQNGKGRKYFHQNSDFYIPKATLKDSGSYFCRGLIGSKNVSSETVNITITQDLAVSSISSFFPPGYQVSFCLVMVLLFAVDTGLYFSMKKSIPSSTRDWEDHKFKWSKDPQDK

SEQ ID NO: 35 - protein, 124 aa, synthetic construct
  source 1..124: note = 34H1
EVQLVESGGGLVQPGGSLRLSCAASGFTFSTYAMYWVRQAPGKGLEWVSTINSDGSSTRYAGSVKGRFTISRDNSKNTLYLQMNSLRAEDTAVYYCAKGWISSPVWGDYVPPVWGQGTMVTVSS

SEQ ID NO: 36 - protein, 124 aa, synthetic construct
  source 1..124: note = 34H2
HVQLVESGGGLVQPGGSLRLSCAASGFTFSTYAMYWVRQAPGKGLEWVSTINSDGSSTRYAGSVKGRFTISRDNSKNTLYLQMNSLRAEDTAVYYCAKGWISSPVWGDYVPPVWGQGTMVTVSS

SEQ ID NO: 37 - protein, 124 aa, synthetic construct
  source 1..124: note = 34H3
EVQLVESGGGLVQPGGSLRLSCAASGFTFSTYAMYWVRQLPGKGLEWVSTINSDGSSTRYAGSVKGRFTISRDNSKNTLYLQMNSLRAEDTAMYYCAKGWISSPVWGDYVPPVWGQGTMVTVSS

SEQ ID NO: 38 - protein, 124 aa, synthetic construct
  source 1..124: note = 34H4
HVQLVESGGGLVQPGGSLRLSCAASGFAFSTYAMYWVRQAPGKGLEWVSTINSDGSSTRYAGSVKGRFTISRDNSKNTLYLQMNSLRAEDTAVYYCAKGWISSPVWGDYVPPVWGQGTMVTVSS

SEQ ID NO: 39 - protein, 124 aa, synthetic construct
  source 1..124: note = 34H5
HVQLVESGGGLVQPGGSLRLSCAASGFAFSTYAMYWVRQLPGKGLEWVSTINSDGSSTRYAGSVKGRFTISRDNSKNTLYLQMNSLRAEDTAMYYCAKGWISSPVWGDYVPPVWGQGTMVTVSS

SEQ ID NO: 40 - protein, 123 aa, synthetic construct
  source 1..123: note = 501V1
EVQLVESGGGVVRPGGSLRLSCAASGFTFDAYPMGWFRQAPGKGLEWVSCINWNGGRTQYGDSVKGRFTISRDNAKNSLYLQMNSLRAEDTALYYCAALYACDSASSPSRRDWGQGTMVTVSS

SEQ ID NO: 41 - protein, 123 aa, synthetic construct
  source 1..123: note = 501V2
EVQLVESGGGVVRPGGSLRLSCAASGFPVDAYPMGWFRQAPGKGLEWVSCINWNGGRTQYGDSVKGRFTISRDNAKNSLYLQMNSLRAEDTALYYCAALYACDSASSPSRRDWGQGTMVTVSS

SEQ ID NO: 42 - protein, 123 aa, synthetic construct
  source 1..123: note = 501V3
EVQLVESGGGVVRPGGSLRLSCAASGFPVDAYPMGWFRQAPGKEREWVSCINWNGGRTQYGDSVKGRFTISRDNAKNSLYLQMNSLRAEDTALYYCAALYACDSASSPSRRDWGQGTMVTVSS

SEQ ID NO: 43 - protein, 123 aa, synthetic construct
  source 1..123: note = 501V3NQ
EVQLVESGGGVVRPGGSLRLSCAASGFPVDAYPMGWFRQAPGKGLEWVSCINWQGGRTQYGDSVKGRFTISRDNAKNSLYLQMNSLRAEDTALYYCAALYACDSASSPSRRDWGQGTMVTVSS

SEQ ID NO: 44 - protein, 17 aa, synthetic construct
  source 1..17: note = CDR
CINWQGGRTQYGDSVKG

SEQ ID NO: 45 - protein, 448 aa, synthetic construct
  source 1..448: note = 1903
EVQLVQSGAEVKKPGASVKVSCKASGYTFTSYWMHWVRQAPGQRLEWMGMIHPNSGSTNYNEKFKGRVTITRDTSASTAYMELSSLRSEDTAVYYCARLKTGNSFDYWGQGTTVTVSSASTKGPSVFPLAPSSKSTSGGTAALGCLVKDYFPEPVTVSWNSGALTSGVHTFPAVLQSSGLYSLSSVVTVPSSSLGTQTYICNVNHKPSNTKVDKKVEPKSCDKTHTCPPCPAPELLGGPDVFLFPPKPKDTLMISRTPEVTCVVVDVSHEDPEVKFNWYVDGVEVHNAKTKPREEQYNSTYRVVSVLTVLHQDWLNGKEYKCKVSNKALPAPEEKTISKAKGQPREPQVYTLPPSRDELTKNQVSLTCLVKGFYPSDIAVEWESNGQPENNYKTTPPVLDSDGSFFLYSKLTVDKSRWQQGNVFSCSVMHEALHNHYTQKSLSLSPGK

SEQ ID NO: 46 - protein, 220 aa, synthetic construct
  source 1..220: note = 1903
DIVLTQSPDSLAVSLGERATINCKSSQSLLNSGNQKNYLTWYQQKPGQPPKLLIYWASTRESGVPDRFSGSGSGTDFTLTISSLQAEDVAVYYCQNAYTYPFTFGQGTKLEIKRTVAAPSVFIFPPSDEQLKSGTASVVCLLNNFYPREAKVQWKVDNALQSGNSQESVTEQDSKDSTYSLSSTLTLSKADYEKHKVYACEVTHQGLSSPVTKSFNRGEC

SEQ ID NO: 47 - protein, 582 aa, synthetic construct
  source 1..582: note = 1903 x C5_V2
EVQLVQSGAEVKKPGASVKVSCKASGYTFTSYWMHWVRQAPGQRLEWMGMIHPNSGSTNYNEKFKGRVTITRDTSASTAYMELSSLRSEDTAVYYCARLKTGNSFDYWGQGTTVTVSSASTKGPSVFPLAPSSKSTSGGTAALGCLVKDYFPEPVTVSWNSGALTSGVHTFPAVLQSSGLYSLSSVVTVPSSSLGTQTYICNVNHKPSNTKVDKKVEPKSCDKTHTCPPCPAPELLGGPDVFLFPPKPKDTLMISRTPEVTCVVVDVSHEDPEVKFNWYVDGVEVHNAKTKPREEQYNSTYRVVSVLTVLHQDWLNGKEYKCKVSNKALPAPEEKTISKAKGQPREPQVYTLPPSRDELTKNQVSLTCLVKGFYPSDIAVEWESNGQPENNYKTTPPVLDSDGSFFLYSKLTVDKSRWQQGNVFSCSVMHEALHNHYTQKSLSLSPGKGGGGSGGGGSQVQLVESGGGLVQPGGSLRLSCSASGFTFSSYAMSWVRQAPGKGLEWVSDINSGGESTFYEDSVKGRFTISRDNAKNTLYLQMNSLRAEDTAVYYCAKHPLTFTIATMNDYDYWGQGTLVTVSS

SEQ ID NO: 48 - protein, 582 aa, synthetic construct
  source 1..582: note = 1903 x C5_V2-YTI
EVQLVQSGAEVKKPGASVKVSCKASGYTFTSYWMHWVRQAPGQRLEWMGMIHPNSGSTNYNEKFKGRVTITRDTSASTAYMELSSLRSEDTAVYYCARLKTGNSFDYWGQGTTVTVSSASTKGPSVFPLAPSSKSTSGGTAALGCLVKDYFPEPVTVSWNSGALTSGVHTFPAVLQSSGLYSLSSVVTVPSSSLGTQTYICNVNHKPSNTKVDKKVEPKSCDKTHTCPPCPAPELLGGPDVFLFPPKPKDTLMISRTPEVTCVVVDVSHEDPEVKFNWYVDGVEVHNAKTKPREEQYNSTYRVVSVLTVLHQDWLNGKEYKCKVSNKALPAPEEKTISKAKGQPREPQVYTLPPSRDELTKNQVSLTCLVKGFYPSDIAVEWESNGQPENNYKTTPPVLDSDGSFFLYSKLTVDKSRWQQGNVFSCSVMHEALHNHYTQKSLSLSPGKGGGGSGGGGSQVQLVESGGGLVQPGGSLRLSCSASGFTFSSYAMSWVRQAPGKGLEWVSDINSGGESTFYEDSVKGRFTISRDNAKNTLYLQMNSLRAEDTAVYYCAKHPLTYTIATMNDYDYWGQGTLVTVSS

SEQ ID NO: 49 - protein, 583 aa, synthetic construct
  source 1..583: note = 1903 x C5_V2-YTI-AA
EVQLVQSGAEVKKPGASVKVSCKASGYTFTSYWMHWVRQAPGQRLEWMGMIHPNSGSTNYNEKFKGRVTITRDTSASTAYMELSSLRSEDTAVYYCARLKTGNSFDYWGQGTTVTVSSASTKGPSVFPLAPSSKSTSGGTAALGCLVKDYFPEPVTVSWNSGALTSGVHTFPAVLQSSGLYSLSSVVTVPSSSLGTQTYICNVNHKPSNTKVDKKVEPKSCDKTHTCPPCPAPELLGGPDVFLFPPKPKDTLMISRTPEVTCVVVDVSHEDPEVKFNWYVDGVEVHNAKTKPREEQYNSTYRVVSVLTVLHQDWLNGKEYKCKVSNKALPAPEEKTISKAKGQPREPQVYTLPPSRDELTKNQVSLTCLVKGFYPSDIAVEWESNGQPENNYKTTPPVLDSDGSFFLYSKLTVDKSRWQQGNVFSCSVMHEALHNHYTQKSLSLSPGKGGGGSGGGGSQVQLVESGGGLVQPGGSLRLSCSASGFTFSSYAMSWVRQAPGKGLEWVSDINSGGESTFYEDSVKGRFTISRDNAKNTLYLQMNSLRAEDTAVYYCAKHPLTYTIATMNDYDYWGQGTLVTVSAA

SEQ ID NO: 50 - protein, 582 aa, synthetic construct; identical to SEQ ID NO: 47
  source 1..582: note = 1903 x C5_V2 x 34H3

SEQ ID NO: 51 - protein, 359 aa, synthetic construct
  source 1..359: note = 1903 x C5_V2 x 34H3
DIVLTQSPDSLAVSLGERATINCKSSQSLLNSGNQKNYLTWYQQKPGQPPKLLIYWASTRESGVPDRFSGSGSGTDFTLTISSLQAEDVAVYYCQNAYTYPFTFGQGTKLEIKRTVAAPSVFIFPPSDEQLKSGTASVVCLLNNFYPREAKVQWKVDNALQSGNSQESVTEQDSKDSTYSLSSTLTLSKADYEKHKVYACEVTHQGLSSPVTKSFNRGECGGGGSGGGGSGGGGSEVQLVESGGGLVQPGGSLRLSCAASGFTFSTYAMYWVRQLPGKGLEWVSTINSDGSSTRYAGSVKGRFTISRDNSKNTLYLQMNSLRAEDTAMYYCAKGWISSPVWGDYVPPVWGQGTMVTVSS

SEQ ID NO: 52 - protein, 582 aa, synthetic construct; identical to SEQ ID NO: 48
  source 1..582: note = 1903 x C5_V2-YTI x 34H3

SEQ ID NO: 53 - protein, 583 aa, synthetic construct; identical to SEQ ID NO: 49
  source 1..583: note = 1903 x C5_V2-YTI x 34H3-AA

SEQ ID NO: 54 - protein, 360 aa, synthetic construct
  source 1..360: note = 1903 x C5_V2-YTI x 34H3-AA
DIVLTQSPDSLAVSLGERATINCKSSQSLLNSGNQKNYLTWYQQKPGQPPKLLIYWASTRESGVPDRFSGSGSGTDFTLTISSLQAEDVAVYYCQNAYTYPFTFGQGTKLEIKRTVAAPSVFIFPPSDEQLKSGTASVVCLLNNFYPREAKVQWKVDNALQSGNSQESVTEQDSKDSTYSLSSTLTLSKADYEKHKVYACEVTHQGLSSPVTKSFNRGECGGGGSGGGGSGGGGSEVQLVESGGGLVQPGGSLRLSCAASGFTFSTYAMYWVRQLPGKGLEWVSTINSDGSSTRYAGSVKGRFTISRDNSKNTLYLQMNSLRAEDTAMYYCAKGWISSPVWGDYVPPVWGQGTMVTVSAA

SEQ ID NO: 55 - protein, 582 aa, synthetic construct
  source 1..582: note = 1903 x C5_V2-LALA
EVQLVQSGAEVKKPGASVKVSCKASGYTFTSYWMHWVRQAPGQRLEWMGMIHPNSGSTNYNEKFKGRVTITRDTSASTAYMELSSLRSEDTAVYYCARLKTGNSFDYWGQGTTVTVSSASTKGPSVFPLAPSSKSTSGGTAALGCLVKDYFPEPVTVSWNSGALTSGVHTFPAVLQSSGLYSLSSVVTVPSSSLGTQTYICNVNHKPSNTKVDKKVEPKSCDKTHTCPPCPAPEAAGGPSVFLFPPKPKDTLMISRTPEVTCVVVDVSHEDPEVKFNWYVDGVEVHNAKTKPREEQYNSTYRVVSVLTVLHQDWLNGKEYKCKVSNKALPAPIEKTISKAKGQPREPQVYTLPPSRDELTKNQVSLTCLVKGFYPSDIAVEWESNGQPENNYKTTPPVLDSDGSFFLYSKLTVDKSRWQQGNVFSCSVMHEALHNHYTQKSLSLSPGKGGGGSGGGGSQVQLVESGGGLVQPGGSLRLSCSASGFTFSSYAMSWVRQAPGKGLEWVSDINSGGESTFYEDSVKGRFTISRDNAKNTLYLQMNSLRAEDTAVYYCAKHPLTFTIATMNDYDYWGQGTLVTVSS

SEQ ID NO: 56 - protein, 582 aa, synthetic construct
  source 1..582: note = 1903 x C5_V2-YTI-LALA
EVQLVQSGAEVKKPGASVKVSCKASGYTFTSYWMHWVRQAPGQRLEWMGMIHPNSGSTNYNEKFKGRVTITRDTSASTAYMELSSLRSEDTAVYYCARLKTGNSFDYWGQGTTVTVSSASTKGPSVFPLAPSSKSTSGGTAALGCLVKDYFPEPVTVSWNSGALTSGVHTFPAVLQSSGLYSLSSVVTVPSSSLGTQTYICNVNHKPSNTKVDKKVEPKSCDKTHTCPPCPAPEAAGGPSVFLFPPKPKDTLMISRTPEVTCVVVDVSHEDPEVKFNWYVDGVEVHNAKTKPREEQYNSTYRVVSVLTVLHQDWLNGKEYKCKVSNKALPAPIEKTISKAKGQPREPQVYTLPPSRDELTKNQVSLTCLVKGFYPSDIAVEWESNGQPENNYKTTPPVLDSDGSFFLYSKLTVDKSRWQQGNVFSCSVMHEALHNHYTQKSLSLSPGKGGGGSGGGGSQVQLVESGGGLVQPGGSLRLSCSASGFTFSSYAMSWVRQAPGKGLEWVSDINSGGESTFYEDSVKGRFTISRDNAKNTLYLQMNSLRAEDTAVYYCAKHPLTYTIATMNDYDYWGQGTLVTVSS

SEQ ID NO: 57 - protein, 5 aa, synthetic construct
  source 1..5: note = CDR
SYWMH

SEQ ID NO: 58 - protein, 17 aa, synthetic construct
  source 1..17: note = CDR
MIHPNSGSTNYNEKFKG

SEQ ID NO: 59 - protein, 9 aa, synthetic construct
  source 1..9: note = CDR
LKTGNSFDY

SEQ ID NO: 60 - protein, 17 aa, synthetic construct
  source 1..17: note = CDR
KSSQSLLNSGNQKNYLT

SEQ ID NO: 61 - protein, 7 aa, synthetic construct
  source 1..7: note = CDR
WASTRES

SEQ ID NO: 62 - protein, 9 aa, synthetic construct
  source 1..9: note = CDR
QNAYTYPFT

SEQ ID NO: 63 - protein, 118 aa, synthetic construct
  source 1..118: note = 1903 VH
EVQLVQSGAEVKKPGASVKVSCKASGYTFTSYWMHWVRQAPGQRLEWMGMIHPNSGSTNYNEKFKGRVTITRDTSASTAYMELSSLRSEDTAVYYCARLKTGNSFDYWGQGTTVTVSS

SEQ ID NO: 64 - protein, 113 aa, synthetic construct
  source 1..113: note = 1903 VL
DIVLTQSPDSLAVSLGERATINCKSSQSLLNSGNQKNYLTWYQQKPGQPPKLLIYWASTRESGVPDRFSGSGSGTDFTLTISSLQAEDVAVYYCQNAYTYPFTFGQGTKLEIK

SEQ ID NO: 65 - protein, 232 aa, synthetic construct
  source 1..232: note = IgG1-Fc
EPKSCDKTHTCPPCPAPELLGGPDVFLFPPKPKDTLMISRTPEVTCVVVDVSHEDPEVKFNWYVDGVEVHNAKTKPREEQYNSTYRVVSVLTVLHQDWLNGKEYKCKVSNKALPAPEEKTISKAKGQPREPQVYTLPPSRDELTKNQVSLTCLVKGFYPSDIAVEWESNGQPENNYKTTPPVLDSDGSFFLYSKLTVDKSRWQQGNVFSCSVMHEALHNHYTQKSLSLSPGK

SEQ ID NO: 66 - protein, 8 aa, synthetic construct
  source 1..8: note = CDR
GFTFSSYA

SEQ ID NO: 67 - protein, 8 aa, synthetic construct
  source 1..8: note = CDR
INSGGEST

SEQ ID NO: 68 - protein, 17 aa, synthetic construct
  source 1..17: note = CDR
AKHPLTFTIATMNDYDY

SEQ ID NO: 69 - protein, 17 aa, synthetic construct
  source 1..17: note = CDR
AKHPLTYTIATMNDYDY

SEQ ID NO: 70 - protein, 7 aa, synthetic construct
  source 1..7: note = CDR
GFTFSSY

SEQ ID NO: 71 - protein, 6 aa, synthetic construct
  source 1..6: note = CDR
NSGGES

SEQ ID NO: 72 - protein, 10 aa, synthetic construct
  source 1..10: note = CDR
GFTFSSYAMS

SEQ ID NO: 73 - protein, 10 aa, synthetic construct
  source 1..10: note = CDR
DINSGGESTF

SEQ ID NO: 74 - protein, 6 aa, synthetic construct
  source 1..6: note = CDR
SSYAMS

SEQ ID NO: 75 - protein, 13 aa, synthetic construct
  source 1..13: note = CDR
WVSDINSGGESTF

SEQ ID NO: 76 - protein, 16 aa, synthetic construct
  source 1..16: note = CDR
AKHPLTFTIATMNDYD

SEQ ID NO: 77 - protein, 16 aa, synthetic construct
  source 1..16: note = CDR
AKHPLTYTIATMNDYD

SEQ ID NO: 78 - protein, 8 aa, synthetic construct
  source 1..8: note = CDR
GYTFTSYW

SEQ ID NO: 79 - protein, 8 aa, synthetic construct
  source 1..8: note = CDR
IHPNSGST

SEQ ID NO: 80 - protein, 11 aa, synthetic construct
  source 1..11: note = CDR
ARLKTGNSFDY

SEQ ID NO: 81 - protein, 12 aa, synthetic construct
  source 1..12: note = CDR
QSLLNSGNQKNY

SEQ ID NO: 82 - protein, 7 aa, synthetic construct
  source 1..7: note = CDR
GYTFTSY

SEQ ID NO: 83 - protein, 6 aa, synthetic construct
  source 1..6: note = CDR
HPNSGS

SEQ ID NO: 84 - protein, 10 aa, synthetic construct
  source 1..10: note = CDR
GYTFTSYWMH

SEQ ID NO: 85 - protein, 10 aa, synthetic construct
  source 1..10: note = CDR
MIHPNSGSTN

SEQ ID NO: 86 - protein, 6 aa, synthetic construct
  source 1..6: note = CDR
TSYWMH

SEQ ID NO: 87 - protein, 13 aa, synthetic construct
  source 1..13: note = CDR
WMGMIHPNSGSTN

SEQ ID NO: 88 - protein, 10 aa, synthetic construct
  source 1..10: note = CDR
ARLKTGNSFD

SEQ ID NO: 89 - protein, 13 aa, synthetic construct
  source 1..13: note = CDR
LNSGNQKNYLTWY

SEQ ID NO: 90 - protein, 10 aa, synthetic construct
  source 1..10: note = CDR
LLIYWASTRE

SEQ ID NO: 91 - protein, 8 aa, synthetic construct
  source 1..8: note = CDR
QNAYTYPF

SEQ ID NO: 92 - protein, 8 aa, synthetic construct
  source 1..8: note = CDR
GFAFSTYA

SEQ ID NO: 93 - protein, 8 aa, synthetic construct
  source 1..8: note = CDR
INSDGSST

SEQ ID NO: 94 - protein, 17 aa, synthetic construct
  source 1..17: note = CDR
AKGWISSPVWGDYVPPV

SEQ ID NO: 95 - protein, 7 aa, synthetic construct
  source 1..7: note = CDR
GFAFSTY

SEQ ID NO: 96 - protein, 6 aa, synthetic construct
  source 1..6: note = CDR
NSDGSS

SEQ ID NO: 97 - protein, 10 aa, synthetic construct
  source 1..10: note = CDR
GFTFSTYAMY

SEQ ID NO: 98 - protein, 10 aa, synthetic construct
  source 1..10: note = CDR
TINSDGSSTR

SEQ ID NO: 99 - protein, 6 aa, synthetic construct
  source 1..6: note = CDR
STYAMY

SEQ ID NO: 100 - protein, 13 aa, synthetic construct
  source 1..13: note = CDR
WVSTINSDGSSTR

SEQ ID NO: 101 - protein, 16 aa, synthetic construct
  source 1..16: note = CDR
AKGWISSPVWGDYVPP

SEQ ID NO: 102 - protein, 5 aa, synthetic construct
  source 1..5: note = G4S
GGGGS

SEQ ID NO: 103 - protein, 10 aa, synthetic construct
  source 1..10: note = (G4S)2
GGGGSGGGGS

SEQ ID NO: 104 - protein, 15 aa, synthetic construct
  source 1..15: note = (G4S)3
GGGGSGGGGSGGGGS

SEQ ID NO: 105 - protein, 20 aa, synthetic construct
  source 1..20: note = (G4S)4
GGGGSGGGGSGGGGSGGGGS

SEQ ID NO: 106 - protein, 25 aa, synthetic construct
  source 1..25: note = (G4S)5
GGGGSGGGGSGGGGSGGGGSGGGGS

SEQ ID NO: 107 - protein, 4 aa, synthetic construct
  source 1..4: note = ASGS
ASGS